European Patent Specification EP 3 612 550 B1, published June 18, 2025. Title: MODIFIED CYTOMEGALOVIRUS PROTEINS AND STABILIZED COMPLEXES. Applicant: GLAXOSMITHKLINE BIOLOGICALS, S.A. The sequence listing filed with the application follows.

SEQUENCE LISTING (83 sequences)

SEQ ID NO: 1 - protein, 742 aa, Artificial Sequence
  HCMV Merlin strain, full length gH
MRPGLPSYLIILAVCLFSHLLSSRYGAEAVSEPLDKAFHLLLNTYGRPIRFLRENTTQCTYNSSLRNSTVVRENAISFNFFQSYNQYYVFHMPRCLFAGPLAEQFLNQVDLTETLERYQQRLNTYALVSKDLASYRSFSQQLKAQDSLGEQPTTVPPPIDLSIPHVWMPPQTTPHGWTESHTTSGLHRPHFNQTCILFDGHDLLFSTVTPCLHQGFYLIDELRYVKITLTEDFFVVTVSIDDDTPMLLIFGHLPRVLFKAPYQRDNFILRQTEKHELLVLVKKDQLNRHSYLKDPDFLDAALDFNYLDLSALLRNSFHRYAVDVLKSGRCQMLDRRTVEMAFAYALALFAAARQEEAGAQVSVPRALDRQAALLQIQEFMITCLSQTPPRTTLLLYPTAVDLAKRALWTPNQITDITSLVRLVYILSKQNQQHLIPQWALRQIADFALKLHKTHLASFLSAFARQELYLMGSLVHSMLVHTTERREIFIVETGLCSLAELSHFTQLLAHPHHEYLSDLYTPCSSSGRRDHSLERLTRLFPDATVPATVPAALSILSTMQPSTLETFPDLFCLPLGESFSALTVSEHVSYIVTNQYLIKGISYPVSTTVVGQSLIITQTDSQTKCELTRNMHTTHSITVALNISLENCAFCQSALLEYDDTQGVINIMYMHDSDDVLFALDPYNEVVVSSPRTHYLMLLKNGTVLEVTDVVVDATDSRLLMMSVYALSAIIGIYLLYRMLKTC

SEQ ID NO: 2 - protein, 719 aa, Artificial Sequence
  HCMV Merlin strain, mature gH
RYGAEAVSEPLDKAFHLLLNTYGRPIRFLRENTTQCTYNSSLRNSTVVRENAISFNFFQSYNQYYVFHMPRCLFAGPLAEQFLNQVDLTETLERYQQRLNTYALVSKDLASYRSFSQQLKAQDSLGEQPTTVPPPIDLSIPHVWMPPQTTPHGWTESHTTSGLHRPHFNQTCILFDGHDLLFSTVTPCLHQGFYLIDELRYVKITLTEDFFVVTVSIDDDTPMLLIFGHLPRVLFKAPYQRDNFILRQTEKHELLVLVKKDQLNRHSYLKDPDFLDAALDFNYLDLSALLRNSFHRYAVDVLKSGRCQMLDRRTVEMAFAYALALFAAARQEEAGAQVSVPRALDRQAALLQIQEFMITCLSQTPPRTTLLLYPTAVDLAKRALWTPNQITDITSLVRLVYILSKQNQQHLIPQWALRQIADFALKLHKTHLASFLSAFARQELYLMGSLVHSMLVHTTERREIFIVETGLCSLAELSHFTQLLAHPHHEYLSDLYTPCSSSGRRDHSLERLTRLFPDATVPATVPAALSILSTMQPSTLETFPDLFCLPLGESFSALTVSEHVSYIVTNQYLIKGISYPVSTTVVGQSLIITQTDSQTKCELTRNMHTTHSITVALNISLENCAFCQSALLEYDDTQGVINIMYMHDSDDVLFALDPYNEVVVSSPRTHYLMLLKNGTVLEVTDVVVDATDSRLLMMSVYALSAIIGIYLLYRMLKTC

SEQ ID NO: 3 - protein, 715 aa, Artificial Sequence
  HCMV Truncated gH, residues 1 to 715 of SEQ ID NO: 1
MRPGLPSYLIILAVCLFSHLLSSRYGAEAVSEPLDKAFHLLLNTYGRPIRFLRENTTQCTYNSSLRNSTVVRENAISFNFFQSYNQYYVFHMPRCLFAGPLAEQFLNQVDLTETLERYQQRLNTYALVSKDLASYRSFSQQLKAQDSLGEQPTTVPPPIDLSIPHVWMPPQTTPHGWTESHTTSGLHRPHFNQTCILFDGHDLLFSTVTPCLHQGFYLIDELRYVKITLTEDFFVVTVSIDDDTPMLLIFGHLPRVLFKAPYQRDNFILRQTEKHELLVLVKKDQLNRHSYLKDPDFLDAALDFNYLDLSALLRNSFHRYAVDVLKSGRCQMLDRRTVEMAFAYALALFAAARQEEAGAQVSVPRALDRQAALLQIQEFMITCLSQTPPRTTLLLYPTAVDLAKRALWTPNQITDITSLVRLVYILSKQNQQHLIPQWALRQIADFALKLHKTHLASFLSAFARQELYLMGSLVHSMLVHTTERREIFIVETGLCSLAELSHFTQLLAHPHHEYLSDLYTPCSSSGRRDHSLERLTRLFPDATVPATVPAALSILSTMQPSTLETFPDLFCLPLGESFSALTVSEHVSYIVTNQYLIKGISYPVSTTVVGQSLIITQTDSQTKCELTRNMHTTHSITVALNISLENCAFCQSALLEYDDTQGVINIMYMHDSDDVLFALDPYNEVVVSSPRTHYLMLLKNGTVLEVTDVVVDATD

SEQ ID NO: 4 - protein, 692 aa, Artificial Sequence
  HCMV mature truncated gH, residues 24 to 715 of SEQ ID NO: 1
RYGAEAVSEPLDKAFHLLLNTYGRPIRFLRENTTQCTYNSSLRNSTVVRENAISFNFFQSYNQYYVFHMPRCLFAGPLAEQFLNQVDLTETLERYQQRLNTYALVSKDLASYRSFSQQLKAQDSLGEQPTTVPPPIDLSIPHVWMPPQTTPHGWTESHTTSGLHRPHFNQTCILFDGHDLLFSTVTPCLHQGFYLIDELRYVKITLTEDFFVVTVSIDDDTPMLLIFGHLPRVLFKAPYQRDNFILRQTEKHELLVLVKKDQLNRHSYLKDPDFLDAALDFNYLDLSALLRNSFHRYAVDVLKSGRCQMLDRRTVEMAFAYALALFAAARQEEAGAQVSVPRALDRQAALLQIQEFMITCLSQTPPRTTLLLYPTAVDLAKRALWTPNQITDITSLVRLVYILSKQNQQHLIPQWALRQIADFALKLHKTHLASFLSAFARQELYLMGSLVHSMLVHTTERREIFIVETGLCSLAELSHFTQLLAHPHHEYLSDLYTPCSSSGRRDHSLERLTRLFPDATVPATVPAALSILSTMQPSTLETFPDLFCLPLGESFSALTVSEHVSYIVTNQYLIKGISYPVSTTVVGQSLIITQTDSQTKCELTRNMHTTHSITVALNISLENCAFCQSALLEYDDTQGVINIMYMHDSDDVLFALDPYNEVVVSSPRTHYLMLLKNGTVLEVTDVVVDATD

SEQ ID NO: 5 - protein, 742 aa, Artificial Sequence
  HCMV Towne strain, full length gH
MRPGLPSYLIVLAVCLLSHLLSSRYGAEAISEPLDKAFHLLLNTYGRPIRFLRENTTQCTYNSSLRNSTVVRENAISFNFFQSYNQYYVFHMPRCLFAGPLAEQFLNQVDLTETLERYQQRLNTYALVSKDLASYRSFSQQLKAQDSLGEQPTTVPPPIDLSIPHVWMPPQTTPHGWTESHTTSGLHRPHFNQTCILFDGHDLLFSTVTPCLHQGFYLIDELRYVKITLTEDFFVVTVSIDDDTPMLLIFGHLPRVLFKAPYQRDNFILRQTEKHELLVLVKKDQLNRHSYLKDPDFLDAALDFNYLDLSALLRNSFHRYAVDVLKSGRCQMLDRRTVEMAFAYALALFAAARQEEAGAQVSVPRALDRQAALLQIQEFMITCLSQTPPRTTLLLYPTAVDLAKRALWTPNQITDITSLVRLVYILSKQNQQHLIPQWALRQIADFALKLHKTHLASFLSAFARQELYLMGSLVHSMLVHTTERREIFIVETGLCSLAELSHFTQLLAHPHHEYLSDLYTPCSSSGRRDHSLERLTRLFPDATVPTTVPAALSILSTMQPSTLETFPDLFCLPLGESFSALTVSEHVSYVVTNQYLIKGISYPVSTTVVGQSLIITQTDSQTKCELTRNMHTTHSITAALNISLENCAFCQSALLEYDDTQGVINIMYMHDSDDVLFALDPYNEVVVSSPRTHYLMLLKNGTVLEVTDVVVDATDSRLLMMSVYALSAIIGIYLLYRMLKTC

SEQ ID NO: 6 - protein, 743 aa, Artificial Sequence
  HCMV AD169 strain, full length gH
MRPGLPPYLTVFTVYLLSHLPSQRYGADAASEALDPHAFHLLLNTYGRPIRFLRENTTQCTYNSSLRNSTVVRENAISFNFFQSYNQYYVFHMPRCLFAGPLAEQFLNQVDLTETLERYQQRLNTYALVSKDLASYRSFSQQLKAQDSLGQQPTTVPPPIDLSIPHVWMPPQTTPHDWKGSHTTSGLHRPHFNQTCILFDGHDLLFSTVTPCLHQGFYLMDELRYVKITLTEDFFVVTVSIDDDTPMLLIFGHLPRVLFKAPYQRDNFILRQTEKHELLVLVKKAQLNRHSYLKDSDFLDAALDFNYLDLSALLRNSFHRYAVDVLKSGRCQMLDRRTVEMAFAYALALFAAARQEEAGTEISIPRALDRQAALLQIQEFMITCLSQTPPRTTLLLYPTAVDLAKRALWTPDQITDITSLVRLVYILSKQNQQHLIPQWALRQIADFALQLHKTHLASFLSAFARQELYLMGSLVHSMLVHTTERREIFIVETGLCSLAELSHFTQLLAHPHHEYLSDLYTPCSSSGRRDHSLERLTRLFPDATVPATVPAALSILSTMQPSTLETFPDLFCLPLGESFSALTVSEHVSYVVTNQYLIKGISYPVSTTVVGQSLIITQTDSQTKCELTRNMHTTHSITAALNISLENCAFCQSALLEYDDTQGVINIMYMHDSDDVLFALDPYNEVVVSSPRTHYLMLLKNGTVLEVTDVVVDATDSRLLMMSVYALSAIIGIYLLYRMLKTC

SEQ ID NO: 7 - protein, 278 aa, Artificial Sequence
  HCMV Merlin strain, full length gL
MCRRPDCGFSFSPGPVILLWCCLLLPIVSSAAVSVAPTAAEKVPAECPELTRRCLLGEVFEGDKYESWLRPLVNVTGRDGPLSQLIRYRPVTPEAANSVLLDEAFLDTLALLYNNPDQLRALLTLLSSDTAPRWMTVMRGYSECGDGSPAVYTCVDDLCRGYDLTRLSYGRSIFTEHVLGFELVPPSLFNVVVAIRNEATRTNRAVRLPVSTAAAPEGITLFYGLYNAVKEFCLRHQLDPPLLRHLDKYYAGLPPELKQTRVNLPAHSRYGPQAVDAR

SEQ ID NO: 8 - protein, 248 aa, Artificial Sequence
  HCMV Merlin strain, mature full length gL
AAVSVAPTAAEKVPAECPELTRRCLLGEVFEGDKYESWLRPLVNVTGRDGPLSQLIRYRPVTPEAANSVLLDEAFLDTLALLYNNPDQLRALLTLLSSDTAPRWMTVMRGYSECGDGSPAVYTCVDDLCRGYDLTRLSYGRSIFTEHVLGFELVPPSLFNVVVAIRNEATRTNRAVRLPVSTAAAPEGITLFYGLYNAVKEFCLRHQLDPPLLRHLDKYYAGLPPELKQTRVNLPAHSRYGPQAVDAR

SEQ ID NO: 9 - protein, 278 aa, Artificial Sequence
  HCMV Merlin strain, full length LSG gL
MCRRPDCGFSFSPGPVILLWCCLLLPIVSSAAVSVAPTAAEKVPAECPELTRRCLLGEVFEGDKYESWLRPLVNVTGRDGPLSQLIRYRPVTPEALSGVLLDEAFLDTLALLYNNPDQLRALLTLLSSDTAPRWMTVMRGYSECGDGSPAVYTCVDDLCRGYDLTRLSYGRSIFTEHVLGFELVPPSLFNVVVAIRNEATRTNRAVRLPVSTAAAPEGITLFYGLYNAVKEFCLRHQLDPPLLRHLDKYYAGLPPELKQTRVNLPAHSRYGPQAVDAR

SEQ ID NO: 10 - protein, 248 aa, Artificial Sequence
  HCMV Merlin strain, mature LSG gL, residues 31 to 278 of SEQ ID NO: 9
AAVSVAPTAAEKVPAECPELTRRCLLGEVFEGDKYESWLRPLVNVTGRDGPLSQLIRYRPVTPEALSGVLLDEAFLDTLALLYNNPDQLRALLTLLSSDTAPRWMTVMRGYSECGDGSPAVYTCVDDLCRGYDLTRLSYGRSIFTEHVLGFELVPPSLFNVVVAIRNEATRTNRAVRLPVSTAAAPEGITLFYGLYNAVKEFCLRHQLDPPLLRHLDKYYAGLPPELKQTRVNLPAHSRYGPQAVDAR

SEQ ID NO: 11 - protein, 278 aa, Artificial Sequence
  HCMV Towne strain, full length gL
MCRRPDCGFSFSPGPVALLWCCLLLPIVSSATVSVAPTVAEKVPAECPELTRRCLLGEVFQGDKYESWLRPLVNVTRRDGPLSQLIRYRPVTPEAANSVLLDDAFLDTLALLYNNPDQLRALLTLLSSDTAPRWMTVMRGYSECGDGSPAVYTCVDDLCRGYDLTRLSYGRSIFTEHVLGFELVPPSLFNVVVAIRNEATRTNRAVRLPVSTAAAPEGITLFYGLYNAVKEFCLRHQLDPPLLRHLDKYYAGLPPELKQTRVNLPAHSRYGPQAVDAR

SEQ ID NO: 12 - protein, 278 aa, Artificial Sequence
  HCMV AD169 strain, full length gL
MCRRPDCGFSFSPGPVVLLWCCLLLPIVSSVAVSVAPTAAEKVPAECPELTRRCLLGEVFQGDKYESWLRPLVNVTRRDGPLSQLIRYRPVTPEAANSVLLDDAFLDTLALLYNNPDQLRALLTLLSSDTAPRWMTVMRGYSECGDGSPAVYTCVDDLCRGYDLTRLSYGRSIFTEHVLGFELVPPSLFNVVVAIRNEATRTNRAVRLPVSTAAAPEGITLFYGLYNAVKEFCLRHQLDPPLLRHLDKYYAGLPPELKQTRVNLPAHSRYGPQAVDAR

SEQ ID NO: 13 - protein, 171 aa, Artificial Sequence
  HCMV Merlin strain, full length pUL128
MSPKDLTPFLTALWLLLGHSRVPRVRAEECCEFINVNHPPERCYDFKMCNRFTVALRCPDGEVCYSPEKTAEIRGIVTTMTHSLTRQVVHNKLTSCNYNPLYLEADGRIRCGKVNDKAQYLLGAAGSVPYRWINLEYDKITRIVGLDQYLESVKKHKRLDVCRAKMGYMLQ

SEQ ID NO: 14 - protein, 144 aa, Artificial Sequence
  HCMV Merlin strain, mature pUL128, residues 28 to 171 of SEQ ID NO: 13
EECCEFINVNHPPERCYDFKMCNRFTVALRCPDGEVCYSPEKTAEIRGIVTTMTHSLTRQVVHNKLTSCNYNPLYLEADGRIRCGKVNDKAQYLLGAAGSVPYRWINLEYDKITRIVGLDQYLESVKKHKRLDVCRAKMGYMLQ

SEQ ID NO: 15 - protein, 171 aa, Artificial Sequence
  HCMV Towne strain, full length pUL128
MSPKNLTPFLTALWLLLGHSRVPRVRAEECCEFINVNHPPERCYDFKMCNRFTVALRCPDGEVCYSPEKTAEIRGIVTTMTHSLTRQVVHNKLTSCNYNPLYLEADGRIRCGKVNDKAQYLLGAAGSVPYRWINLEYDKITRIVGLDQYLESVKKHKRLDVCRAKMGYMLQ

SEQ ID NO: 16 - protein, 171 aa, Artificial Sequence
  HCMV AD169 strain, full length pUL128
MSPKDLTPFLTTLWLLLGHSRVPRVRAEECCEFINVNHPPERCYDFKMCNRFTVALRCPDGEVCYSPEKTAEIRGIVTTMTHSLTRQVVHNKLTSCNYNPLYLEADGRIRCGKVNDKAQYLLGAAGSVPYRWINLEYDKITRIVGLDQYLESVKKHKRLDVCRAKMGYMLQ

SEQ ID NO: 17 - protein, 214 aa, Artificial Sequence
  HCMV Merlin strain, full length pUL130
MLRLLLRHHFHCLLLCAVWATPCLASPWSTLTANQNPSPPWSKLTYSKPHDAATFYCPFLYPSPPRSPLQFSGFQRVSTGPECRNETLYLLYNREGQTLVERSSTWVKKVIWYLSGRNQTILQRMPRTASKPSDGNVQISVEDAKIFGAHMVPKQTKLLRFVVNDGTRYQMCVMKLESWAHVFRDYSVSFQVRLTFTEANNQTYTFCTHPNLIV

SEQ ID NO: 18 - protein, 189 aa, Artificial Sequence
  HCMV Merlin strain, mature pUL130, residues 26 to 214 of SEQ ID NO: 17
SPWSTLTANQNPSPPWSKLTYSKPHDAATFYCPFLYPSPPRSPLQFSGFQRVSTGPECRNETLYLLYNREGQTLVERSSTWVKKVIWYLSGRNQTILQRMPRTASKPSDGNVQISVEDAKIFGAHMVPKQTKLLRFVVNDGTRYQMCVMKLESWAHVFRDYSVSFQVRLTFTEANNQTYTFCTHPNLIV

SEQ ID NO: 19 - protein, 229 aa, Artificial Sequence
  HCMV Towne strain, full length pUL130
MLRLLLRHHFHCLLLCAVWATPCLASPWSTLTANQNPSPPWSKLTYSKPHDAATFYCPFLYPSPPRSPLQFSGFQRVLTGPECRNETLYLLYNREGQTLVERSSTWVKKVIWYLSGRNQTILQRMPRTASKPSDGNVQISVEDAKIFGAHMVPKQTKLLRFVVNDGTRYQMCVMKLESWAHVFRDYSVSFQVRLTFTEANNQTFTPSAPIPISSFEPVARAGNFENRAS

SEQ ID NO: 20 - protein, 214 aa, Artificial Sequence
  HCMV AD169 strain, full length pUL130
MLRLLLRHHFHCLLLCAVWATPCLASPWSTLTANQNPSPPWSKLTYSKPHDAATFYCPFLYPSPPRSPLQFSGFQQVSTGPECRNETLYLLYNREGQTLVERSSTWVKKVIWYLSGRNQTILQRMPQTASKPSDGNVQISVEDAKIFGAHMVPKQTKLLRFVVNDGTRYQMCVMKLESWAHVFRDYSVSFQVRLTFTEANNQTYTFCTHPNLIV

SEQ ID NO: 21 - protein, 129 aa, Artificial Sequence
  HCMV Merlin strain, full length pUL131A
MRLCRVWLSVCLCAVVLGQCQRETAEKNDYYRVPHYWDACSRALPDQTRYKYVEQLVDLTLNYHYDASHGLDNFDVLKRINVTEVSLLISDFRRQNRRGGTNKRTTFNAAGSLAPHARSLEFSVRLFAN

SEQ ID NO: 22 - protein, 111 aa, Artificial Sequence
  HCMV Merlin strain, mature pUL131A, residues 19 to 129 of SEQ ID NO: 21
QCQRETAEKNDYYRVPHYWDACSRALPDQTRYKYVEQLVDLTLNYHYDASHGLDNFDVLKRINVTEVSLLISDFRRQNRRGGTNKRTTFNAAGSLAPHARSLEFSVRLFAN

SEQ ID NO: 23 - protein, 129 aa, Artificial Sequence; identical to SEQ ID NO: 21
  HCMV Towne strain, full length pUL131A

SEQ ID NO: 24 - protein, 74 aa, Artificial Sequence
  HCMV AD169 strain, full length pUL131A
MRLCRVWLSVCLCAVVLGQCQRETAEKKRLLPSTALLGRVLSRAARPNPLQVCGTARGPHVELPLRCEPRLGQL

SEQ ID NO: 25 - protein, 472 aa, Artificial Sequence
  HCMV Merlin strain, full length gO
MGKKEMIMVKGIPKIMLLISITFLLLSLINCNVLVNSRGTRRSWPYTVLSYRGKEILKKQKEDILKRLMSTSSDGYRFLMYPSQQKFHAIVISMDKFPQDYILAGPIRNDSITHMWFDFYSTQLRKPAKYVYSEYNHTAHKITLRPPPCGTVPSMNCLSEMLNVSKRNDTGEKGCGNFTTFNPMFFNVPRWNTKLYIGSNKVNVDSQTIYFLGLTALLLRYAQRNCTRSFYLVNAMSRNLFRVPKYINGTKLKNTMRKLKRKQALVKEQPQKKNKKSQSTTTPYLSYTTSTAFNVTTNVTYSATAAVTRVATSTTGYRPDSNFMKSIMATQLRDLATWVYTTLRYRNEPFCKPDRNRTAVSEFMKNTHVLIRNETPYTIYGTLDMSSLYYNETMSVENETASDNNETTPTSPSTRFQRTFIDPLWDYLDSLLFLDKIRNFSLQLPAYGNLTPPEHRRAANLSTLNSLWWWSQ

SEQ ID NO: 26 - protein, 442 aa, Artificial Sequence
  HCMV Merlin strain, mature gO, residues 31 to 472 of SEQ ID NO: 25
CNVLVNSRGTRRSWPYTVLSYRGKEILKKQKEDILKRLMSTSSDGYRFLMYPSQQKFHAIVISMDKFPQDYILAGPIRNDSITHMWFDFYSTQLRKPAKYVYSEYNHTAHKITLRPPPCGTVPSMNCLSEMLNVSKRNDTGEKGCGNFTTFNPMFFNVPRWNTKLYIGSNKVNVDSQTIYFLGLTALLLRYAQRNCTRSFYLVNAMSRNLFRVPKYINGTKLKNTMRKLKRKQALVKEQPQKKNKKSQSTTTPYLSYTTSTAFNVTTNVTYSATAAVTRVATSTTGYRPDSNFMKSIMATQLRDLATWVYTTLRYRNEPFCKPDRNRTAVSEFMKNTHVLIRNETPYTIYGTLDMSSLYYNETMSVENETASDNNETTPTSPSTRFQRTFIDPLWDYLDSLLFLDKIRNFSLQLPAYGNLTPPEHRRAANLSTLNSLWWWSQ

SEQ ID NO: 27 - protein, 457 aa, Artificial Sequence
  HCMV Towne strain, full length gO
MGRKGEMRGVFNLFFLMSLTFLLFSFINCKIAVARFRVKSQKAKEEERQLKLRILQELASKTGDYYKFFTFPSQQKLYNITVEMKQFPPNSILAGPIRNHSITHLWFDFHTTQLRKPAKYVYSEYNHTGQKITFRPPSCGTIPSMTCLSEMLNVSRRNNTGEENCGNFTTFNPMFFNVPRWNTKLYVGPSKVNVDSQTIYFLGLAALLLRYAQRNCTRSFYLVNAMSRNIFRVPKYINSTKLKNTMRKLKRKQAPVKSISKKSRVSTTTPYSSYTSTIFNVSTNVTYSPIVPTRIPTSTIGYRPDENFMKSILTTQLKDLATWVYTTLRYRDEPFCKPNRNRTAVSEFMKNTHVLIRNETPYTIYGTLDMSSLYYNDTMPVENETASDNNKTTPTSPSTRFQRTFIDPMWDYLDSLLFLSEIRNFSLQSSTYGNLTPPEHRRAVNLSTLNSLWWWLQ

SEQ ID NO: 28 - protein, 466 aa, Artificial Sequence
  HCMV AD169 strain, full length gO
MGRKEMMVRDVPKMVFLISISFLLVSFINCKVMSKALYNRPWRGLVLSKIGKYKLDQLKLEILRQLETTISTKYNVSKQPVKNLTMNMTEFPQYYILAGPIQNYSITYLWFDFYSTQLRKPAKYVYSQYNHTAKTITFRPPPCGTVPSMTCLSEMLNVSKRNDTGEQGCGNFTTFNPMFFNVPRWNTKLYVGPTKVNVDSQTIYFLGLTALLLRYAQRNCTHSFYLVNAMSRNLFRVPKYINGTKLKNTMRKLKRKQAPVKEQFEKKAKKTQSTTTPYFSYTTSAALNVTTNVTYSITTAARRVSTSTIAYRPDSSFMKSIMATQLRDLATWVYTTLRYRQNPFCEPSRNRTAVSEFMKNTHVLIRNETPYTIYGTLDMSSLYYNETMFVENKTASDSNKTTPTSPSMGFQRTFIDPLWDYLDSLLFLDEIRNFSLRSPTYVNLTPPEHRRAVNLSTLNSLWWWLQ

SEQ ID NO: 29 - protein, 278 aa, Artificial Sequence
  HCMV Merlin strain, full length IDG gL
MCRRPDCGFSFSPGPVILLWCCLLLPIVSSAAVSVAPTAAEKVPAECPELTRRCLLGEVFEGDKYESWLRPLVNVTGRDGPLSQLIRYRPVTPEAIDGVLLDEAFLDTLALLYNNPDQLRALLTLLSSDTAPRWMTVMRGYSECGDGSPAVYTCVDDLCRGYDLTRLSYGRSIFTEHVLGFELVPPSLFNVVVAIRNEATRTNRAVRLPVSTAAAPEGITLFYGLYNAVKEFCLRHQLDPPLLRHLDKYYAGLPPELKQTRVNLPAHSRYGPQAVDAR

SEQ ID NO: 30 - protein, 248 aa, Artificial Sequence
  HCMV Merlin strain, mature IDG gL, residues 31 to 278 of SEQ ID NO: 29
AAVSVAPTAAEKVPAECPELTRRCLLGEVFEGDKYESWLRPLVNVTGRDGPLSQLIRYRPVTPEAIDGVLLDEAFLDTLALLYNNPDQLRALLTLLSSDTAPRWMTVMRGYSECGDGSPAVYTCVDDLCRGYDLTRLSYGRSIFTEHVLGFELVPPSLFNVVVAIRNEATRTNRAVRLPVSTAAAPEGITLFYGLYNAVKEFCLRHQLDPPLLRHLDKYYAGLPPELKQTRVNLPAHSRYGPQAVDAR

SEQ ID NO: 31 - DNA, 2229 bp, Artificial Sequence
  Encodes full length gH sequence SEQ ID NO: 1
atgcggccaggcctcccctcctacctcatcatcctcgccgtctgtctcttcagccacctactttcgtcacgatatggcgcagaagccgtatccgaaccgctggacaaagcgtttcacctactgctcaacacctacgggagacccatccgcttcctgcgtgaaaataccacccagtgtacctacaacagcagcctccgtaacagcacggtcgtcagggaaaacgccatcagtttcaactttttccaaagctataatcaatactatgtattccatatgcctcgatgtctttttgcgggtcctctggcggagcagtttctgaaccaggtagatctgaccgaaaccctggaaagataccaacagagacttaacacttacgcgctggtatccaaagacctggccagctaccgatctttttcgcagcagctaaaggcacaagacagcctaggtgaacagcccaccactgtgccaccgcccattgacctgtcaatacctcacgtttggatgccaccgcaaaccactccacacggctggacagaatcacataccacctcaggactacaccgaccacactttaaccagacctgtatcctctttgatggacacgatctactattcagcaccgtcacaccttgtttgcaccaaggcttttacctcatcgacgaactacgttacgttaaaataacactgaccgaggacttcttcgtagttacggtgtccatagacgacgacacacccatgctgcttatcttcggccatcttccacgcgtacttttcaaagcgccctatcaacgcgacaactttatactacgacaaactgaaaaacacgagctcctggtgctagttaagaaagatcaactgaaccgtcactcttatctcaaagacccggactttcttgacgccgcacttgacttcaactacctagacctcagcgcactactacgtaacagctttcaccgttacgccgtggatgtactcaagagcggtcgatgtcagatgctggaccgccgcacggtagaaatggccttcgcctacgcattagcactgttcgcagcagcccgacaagaagaggccggcgcccaagtctccgtcccacgggccctagaccgccaggccgcactcttacaaatacaagaatttatgatcacctgcctctcacaaacaccaccacgcaccacgttgctgctgtatcccacggccgtggacctggccaaacgagccctttggacaccgaatcagatcaccgacatcaccagcctcgtacgcctggtctacatactctctaaacagaatcagcaacatctcatcccccaatgggcactacgacagatcgccgactttgccctaaaactacacaaaacgcacctggcctcttttctttcagccttcgcacgccaagaactctacctcatgggcagcctcgtccactccatgctggtacatacgacggagagacgcgaaatcttcatcgtagaaacgggcctctgttcattggccgagctatcacactttacgcagttgttagctcatccacaccacgaatacctcagcgacctgtacacaccctgttccagtagcgggcgacgcgatcactcgctcgaacgcctcacgcgtctcttccccgatgccaccgtccccgctaccgttcccgccgccctctccatcctatctaccatgcaaccaagcacgctggaaaccttccccgacctgttttgcttgccgctcggcgaatccttctccgcgctgaccgtctccgaacacgtcagttatatcgtaacaaaccagtacctgatcaaaggtatctcctaccctgtctccaccaccgtcgtaggccagagcctcatcatcacccagacggacagtcaaactaaatgcgaactgacgcgcaacatgcataccacacacagcatcacagtggcgctcaacatttcgctagaaaactgcgccttttgccaaagcgccctgctagaatacgacgacacgcaaggcgtcatcaacatcatgtacatgcacgactcggacgacgtccttttcgccctggatccctacaacgaagtggtggtctcatctccgcgaactcactacctcatgcttttgaaaaacggtacggtactagaagtaactgacgtcgtcgtggacgccaccgacagtcgtctcctcatgatgtccgtctacgcgctatcggccatcatcggcatctatctgctctaccgcatgctcaagacatgctga

SEQ ID NO: 32 - DNA, 2145 bp, Artificial Sequence
  Encodes truncated gH sequence SEQ ID NO: 3, is codon optimized for mammal
atgaggcctggcctgccctcctacctgatcatcctggccgtgtgcctgttcagccacctgctgtccagcagatacggcgccgaggccgtgagcgagcccctggacaaggctttccacctgctgctgaacacctacggcagacccatccggtttctgcgggagaacaccacccagtgcacctacaacagcagcctgcggaacagcaccgtcgtgagagagaacgccatcagcttcaactttttccagagctacaaccagtactacgtgttccacatgcccagatgcctgtttgccggccctctggccgagcagttcctgaaccaggtggacctgaccgagacactggaaagataccagcagcggctgaatacctacgccctggtgtccaaggacctggccagctaccggtcctttagccagcagctcaaggctcaggatagcctcggcgagcagcctaccaccgtgccccctcccatcgacctgagcatcccccacgtgtggatgcctccccagaccacccctcacggctggaccgagagccacaccacctccggcctgcacagaccccacttcaaccagacctgcatcctgttcgacggccacgacctgctgtttagcaccgtgaccccctgcctgcaccagggcttctacctgatcgacgagctgagatacgtgaagatcaccctgaccgaggatttcttcgtggtcaccgtgtccatcgacgacgacacccccatgctgctgatcttcggccacctgcccagagtgctgttcaaggccccctaccagcgggacaacttcatcctgcggcagaccgagaagcacgagctgctggtgctggtcaagaaggaccagctgaaccggcactcctacctgaaggaccccgacttcctggacgccgccctggacttcaactacctggacctgagcgccctgctgagaaacagcttccacagatacgccgtggacgtgctgaagtccggacggtgccagatgctcgatcggcggaccgtggagatggccttcgcctatgccctcgccctgttcgccgctgccagacaggaagaggctggcgcccaggtgtcagtgcccagagccctggatagacaggccgccctgctgcagatccaggaattcatgatcacctgcctgagccagaccccccctagaaccaccctgctgctgtaccccacagccgtggatctggccaagagggccctgtggacccccaaccagatcaccgacatcacaagcctcgtgcggctcgtgtacatcctgagcaagcagaaccagcagcacctgatcccccagtgggccctgagacagatcgccgacttcgccctgaagctgcacaagacccatctggccagctttctgagcgccttcgccaggcaggaactgtacctgatgggcagcctggtccacagcatgctggtgcataccaccgagcggcgggagatcttcatcgtggagacaggcctgtgtagcctggccgagctgtcccactttacccagctgctggcccaccctcaccacgagtacctgagcgacctgtacaccccctgcagcagcagcggcagacgggaccacagcctggaacggctgaccagactgttccccgatgccaccgtgcctgctacagtgcctgccgccctgtccatcctgtccaccatgcagcccagcaccctggaaaccttccccgacctgttctgcctgcccctgggcgagagctttagcgccctgaccgtgtccgagcacgtgtcctacatcgtgaccaatcagtacctgatcaagggcatcagctaccccgtgtccaccacagtcgtgggccagagcctgatcatcacccagaccgacagccagaccaagtgcgagctgacccggaacatgcacaccacacacagcatcaccgtggccctgaacatcagcctggaaaactgcgctttctgtcagtctgccctgctggaatacgacgatacccagggcgtgatcaacatcatgtacatgcacgacagcgacgacgtgctgttcgccctggacccctacaacgaggtggtggtgtccagcccccggacccactacctgatgctgctgaagaacggcaccgtgctggaagtgaccgacgtggtggtggacgccaccgac

SEQ ID NO: 33 - DNA, 834 bp, Artificial Sequence
  Encodes full length gL sequence SEQ ID NO: 7
atgtgcagacggcccgactgcggcttcagcttctcccctggacccgtgatcctgctgtggtgctgcctgctgctgcctatcgtgtcctctgccgccgtgtccgtggcccctaccgctgctgagaaggtgcccgccgagtgccctgagctgaccagacgctgtctgctgggcgaggtgttcgagggcgataagtacgagtcctggctgcggcccctggtgaacgtgaccggcagagatggccccctgtcccagctgatccggtacagacctgtgacccccgaggccgccaactccgtgctgctggacgaggcctttctggacaccctggccctgctgtacaacaaccccgaccagctgcgggccctgctgaccctgctgtctagcgacaccgcccctcggtggatgaccgtgatgcggggctactctgagtgcggcgacggctcccctgccgtgtacacctgtgtggacgacctgtgccggggctacgacctgaccagactgtcctacggccggtctatcttcacagagcacgtgctgggcttcgagctggtgcccccctccctgttcaatgtggtggtggctatccggaacgaggccacccggaccaatagagccgtgcggctgcctgtgtctaccgccgctgctcctgagggaatcaccctgttctacggcctgtacaacgccgtgaaagagttctgcctgagacaccagctggacccccctctgctgcggcacctggacaagtactacgccggcctgccccccgagctgaagcagaccagagtgaacctgcccgcccacagcagatacggcccccaggctgtggacgccagg

SEQ ID NO: 34 - DNA, 834 bp, Artificial Sequence
  Encodes full length LSG gL sequence SEQ ID NO: 9
atgtgcagacggcccgactgcggcttcagcttctcccctggacccgtgatcctgctgtggtgctgcctgctgctgcctatcgtgtcctctgccgccgtgtccgtggcccctaccgctgctgagaaggtgcccgccgagtgccctgagctgaccagacgctgtctgctgggcgaggtgttcgagggcgataagtacgagtcctggctgcggcccctggtgaacgtgaccggcagagatggccccctgtcccagctgatccggtacagacctgtgacccccgaggccctgagcggcgtgctgctggacgaggcctttctggacaccctggccctgctgtacaacaaccccgaccagctgcgggccctgctgaccctgctgtctagcgacaccgcccctcggtggatgaccgtgatgcggggctactctgagtgcggcgacggctcccctgccgtgtacacctgtgtggacgacctgtgccggggctacgacctgaccagactgtcctacggccggtctatcttcacagagcacgtgctgggcttcgagctggtgcccccctccctgttcaatgtggtggtggctatccggaacgaggccacccggaccaatagagccgtgcggctgcctgtgtctaccgccgctgctcctgagggaatcaccctgttctacggcctgtacaacgccgtgaaagagttctgcctgagacaccagctggacccccctctgctgcggcacctggacaagtactacgccggcctgccccccgagctgaagcagaccagagtgaacctgcccgcccacagcagatacggcccccaggctgtggacgccagg

SEQ ID NO: 35 - DNA, 834 bp, Artificial Sequence
  Encodes full length IDG gL sequence SEQ ID NO: 29
atgtgcagacggcccgactgcggcttcagcttctcccctggacccgtgatcctgctgtggtgctgcctgctgctgcctatcgtgtcctctgccgccgtgtccgtggcccctaccgctgctgagaaggtgcccgccgagtgccctgagctgaccagacgctgtctgctgggcgaggtgttcgagggcgataagtacgagtcctggctgcggcccctggtgaacgtgaccggcagagatggccccctgtcccagctgatccggtacagacctgtgacccccgaggccatcgatggcgtgctgctggacgaggcctttctggacaccctggccctgctgtacaacaaccccgaccagctgcgggccctgctgaccctgctgtctagcgacaccgcccctcggtggatgaccgtgatgcggggctactctgagtgcggcgacggctcccctgccgtgtacacctgtgtggacgacctgtgccggggctacgacctgaccagactgtcctacggccggtctatcttcacagagcacgtgctgggcttcgagctggtgcccccctccctgttcaatgtggtggtggctatccggaacgaggccacccggaccaatagagccgtgcggctgcctgtgtctaccgccgctgctcctgagggaatcaccctgttctacggcctgtacaacgccgtgaaagagttctgcctgagacaccagctggacccccctctgctgcggcacctggacaagtactacgccggcctgccccccgagctgaagcagaccagagtgaacctgcccgcccacagcagatacggcccccaggctgtggacgccagg

SEQ ID NO: 36 - DNA, 513 bp, Artificial Sequence
  Encodes full length pUL128 sequence SEQ ID NO: 13
atgtcccccaaggacctgacccccttcctgaccaccctgtggctgctgctgggccactctagggtgcccagagtgcgggccgaagagtgctgcgagtttatcaacgtgaaccacccccccgagcggtgctacgacttcaagatgtgcaaccggttcaccgtggccctgcggtgccctgacggcgaagtgtgctactcccccgaaaagaccgccgagatccggggaatcgtgaccacaatgacccactccctgaccagacaggtggtgcacaacaagctgaccagctgcaactacaaccccctgtacctggaagccgacggccggatccgctgcggcaaagtgaacgacaaggcccagtacctgctgggcgctgccggctctgtgccctaccggtggatcaacctggaatacgacaagatcacccggatcgtgggcctggaccagtacctggaatccgtgaagaagcacaagcggctggacgtgtgccgggccaagatgggctatatgctgcag

SEQ ID NO: 37 - DNA, 642 bp, Artificial Sequence
  Encodes full length pUL130 sequence SEQ ID NO: 17
atgctgcggctgctgctgcggcaccacttccactgcctgctgctgtgtgccgtgtgggccaccccttgtctggcctccccgtggtccaccctgaccgccaaccagaaccccagccccccctggtccaagctgacctactccaagcctcacgacgccgctaccttctactgccccttcctgtacccctccccaccccggtccccactgcagttctccggcttccagagagtgtccaccggccctgagtgccggaacgagacactgtacctgctgtacaaccgcgagggccagaccctggtggaacggtcctccacctgggtgaaaaaagtgatctggtatctgtccggccggaaccagacaatcctgcagcggatgcctcggaccgcctccaagccttccgacggcaacgtgcagatctccgtggaagatgccaagatcttcggcgcccacatggtgcccaagcagaccaagctgctgagattcgtggtgaacgacggcacccgctaccagatgtgcgtgatgaagctggaatcctgggcccacgtgttccgggactactcagtgagcttccaagtccgactgaccttcaccgaggccaacaaccagacctacaccttctgcacccaccccaacctgatcgtg

SEQ ID NO: 38 - DNA, 387 bp, Artificial Sequence
  Encodes full length pUL131A sequence SEQ ID NO: 21
atgcggctgtgcagagtgtggctgtccgtgtgcctgtgcgccgtggtgctgggccagtgccagagagagacagccgagaagaacgactactaccgggtgccccactactgggacgcctgctccagagccctgcccgaccagacccggtacaaatacgtggaacagctggtggacctgaccctgaactaccactacgacgcctcccacggcctggacaacttcgacgtgctgaagcggatcaacgtgaccgaggtgtccctgctgatctccgacttccggcggcagaacagaagaggcggcaccaacaagcggaccaccttcaacgccgctggctccctggcccctcacgcccggtccctggaattctctgtgcggctgttcgccaac

SEQ ID NO: 39 - DNA, 1395 bp, Artificial Sequence
  Encoding full length gO sequence SEQ ID NO: 25
atggggaaaaaagagatgataatggtgaaaggcattcctaaaattatgctcctgatctctataacgttcttgctcctttccctcataaattgtaatgtattggtaaactccagaggaacaagacgttcctggccgtataccgtgctatcttatcgaggtaaagagattctgaagaaacagaaggaagatatcttaaaacgattgatgtctacatcatctgacggataccggtttttaatgtaccccagtcagcaaaaatttcatgccatcgttattagcatggataaatttcctcaagactacattttagcgggtcccattagaaatgatagcattacccatatgtggtttgacttttacagtactcaactccgaaaaccagccaagtacgtatattccgaatataatcacacggcccacaaaataacgttacgacccccaccttgcggcacagtgccttctatgaactgcctatccgaaatgttaaatgtttccaaacgcaatgataccggcgaaaaaggttgcggtaatttcaccacgtttaatcctatgtttttcaacgtaccacgttggaacacaaaactgtacataggttccaacaaagtcaacgtggatagtcagacaatctactttttgggcctaaccgccctacttttacgatacgcgcaacgtaactgcactcgcagtttctacctggttaacgccatgagccgaaatttattccgcgttcccaagtatattaacggcaccaagttgaaaaacactatgcgaaaactcaaacgtaaacaagcgcttgtcaaagaacaaccacaaaaaaagaataagaaatctcaaagtactactacgccatatctttcctatacaacgtctaccgctttcaacgtcaccactaacgtgacttatagtgctaccgctgctgtaacgcgggttgccacatctacgacaggttatcgtcctgatagtaactttatgaaatccattatggccacgcagttaagagatctcgcaacatgggtatatactactctgcggtatcggaatgaacccttttgtaaaccagaccgtaaccgtaccgccgtgtcagaatttatgaaaaacacgcacgtactgattcgtaacgaaacgccgtacactatttatggcactcttgacatgagctccttatattacaacgaaaccatgtccgtggaaaacgaaacggcttccgataataacgaaactacacctacgtcaccatcgacgaggtttcagagaacgttcatagatcccctatgggactatctagactcgctgctgtttctagataaaatccgtaactttagcctccagttacccgcgtatggaaatcttaccccgccggaacaccgccgggctgcaaatctatccaccctcaat

SEQ ID NO: 40 - protein, 715 aa, Artificial Sequence
  gH G358R mutant
MRPGLPSYLIILAVCLFSHLLSSRYGAEAVSEPLDKAFHLLLNTYGRPIRFLRENTTQCTYNSSLRNSTVVRENAISFNFFQSYNQYYVFHMPRCLFAGPLAEQFLNQVDLTETLERYQQRLNTYALVSKDLASYRSFSQQLKAQDSLGEQPTTVPPPIDLSIPHVWMPPQTTPHGWTESHTTSGLHRPHFNQTCILFDGHDLLFSTVTPCLHQGFYLIDELRYVKITLTEDFFVVTVSIDDDTPMLLIFGHLPRVLFKAPYQRDNFILRQTEKHELLVLVKKDQLNRHSYLKDPDFLDAALDFNYLDLSALLRNSFHRYAVDVLKSGRCQMLDRRTVEMAFAYALALFAAARQEEARAQVSVPRALDRQAALLQIQEFMITCLSQTPPRTTLLLYPTAVDLAKRALWTPNQITDITSLVRLVYILSKQNQQHLIPQWALRQIADFALKLHKTHLASFLSAFARQELYLMGSLVHSMLVHTTERREIFIVETGLCSLAELSHFTQLLAHPHHEYLSDLYTPCSSSGRRDHSLERLTRLFPDATVPATVPAALSILSTMQPSTLETFPDLFCLPLGESFSALTVSEHVSYIVTNQYLIKGISYPVSTTVVGQSLIITQTDSQTKCELTRNMHTTHSITVALNISLENCAFCQSALLEYDDTQGVINIMYMHDSDDVLFALDPYNEVVVSSPRTHYLMLLKNGTVLEVTDVVVDATD

SEQ ID NO: 41 - protein, 692 aa, Artificial Sequence
  mature gH G358R mutant
RYGAEAVSEPLDKAFHLLLNTYGRPIRFLRENTTQCTYNSSLRNSTVVRENAISFNFFQSYNQYYVFHMPRCLFAGPLAEQFLNQVDLTETLERYQQRLNTYALVSKDLASYRSFSQQLKAQDSLGEQPTTVPPPIDLSIPHVWMPPQTTPHGWTESHTTSGLHRPHFNQTCILFDGHDLLFSTVTPCLHQGFYLIDELRYVKITLTEDFFVVTVSIDDDTPMLLIFGHLPRVLFKAPYQRDNFILRQTEKHELLVLVKKDQLNRHSYLKDPDFLDAALDFNYLDLSALLRNSFHRYAVDVLKSGRCQMLDRRTVEMAFAYALALFAAARQEEARAQVSVPRALDRQAALLQIQEFMITCLSQTPPRTTLLLYPTAVDLAKRALWTPNQITDITSLVRLVYILSKQNQQHLIPQWALRQIADFALKLHKTHLASFLSAFARQELYLMGSLVHSMLVHTTERREIFIVETGLCSLAELSHFTQLLAHPHHEYLSDLYTPCSSSGRRDHSLERLTRLFPDATVPATVPAALSILSTMQPSTLETFPDLFCLPLGESFSALTVSEHVSYIVTNQYLIKGISYPVSTTVVGQSLIITQTDSQTKCELTRNMHTTHSITVALNISLENCAFCQSALLEYDDTQGVINIMYMHDSDDVLFALDPYNEVVVSSPRTHYLMLLKNGTVLEVTDVVVDATD

SEQ ID NO: 42 - protein, 278 aa, Artificial Sequence
  gL N74Q mutant
MCRRPDCGFSFSPGPVILLWCCLLLPIVSSAAVSVAPTAAEKVPAECPELTRRCLLGEVFEGDKYESWLRPLVQVTGRDGPLSQLIRYRPVTPEALSGVLLDEAFLDTLALLYNNPDQLRALLTLLSSDTAPRWMTVMRGYSECGDGSPAVYTCVDDLCRGYDLTRLSYGRSIFTEHVLGFELVPPSLFNVVVAIRNEATRTNRAVRLPVSTAAAPEGITLFYGLYNAVKEFCLRHQLDPPLLRHLDKYYAGLPPELKQTRVNLPAHSRYGPQAVDAR

SEQ ID NO: 43 - protein, 248 aa, Artificial Sequence
  mature gL N74Q mutant
AAVSVAPTAAEKVPAECPELTRRCLLGEVFEGDKYESWLRPLVQVTGRDGPLSQLIRYRPVTPEALSGVLLDEAFLDTLALLYNNPDQLRALLTLLSSDTAPRWMTVMRGYSECGDGSPAVYTCVDDLCRGYDLTRLSYGRSIFTEHVLGFELVPPSLFNVVVAIRNEATRTNRAVRLPVSTAAAPEGITLFYGLYNAVKEFCLRHQLDPPLLRHLDKYYAGLPPELKQTRVNLPAHSRYGPQAVDAR

SEQ ID NO: 44 - protein, 278 aa, Artificial Sequence
  gL G140F mutant
MCRRPDCGFSFSPGPVILLWCCLLLPIVSSAAVSVAPTAAEKVPAECPELTRRCLLGEVFEGDKYESWLRPLVNVTGRDGPLSQLIRYRPVTPEALSGVLLDEAFLDTLALLYNNPDQLRALLTLLSSDTAPRWMTVMRFYSECGDGSPAVYTCVDDLCRGYDLTRLSYGRSIFTEHVLGFELVPPSLFNVVVAIRNEATRTNRAVRLPVSTAAAPEGITLFYGLYNAVKEFCLRHQLDPPLLRHLDKYYAGLPPELKQTRVNLPAHSRYGPQAVDAR

SEQ ID NO: 45 - protein, 248 aa, Artificial Sequence
  mature gL G140F mutant
AAVSVAPTAAEKVPAECPELTRRCLLGEVFEGDKYESWLRPLVNVTGRDGPLSQLIRYRPVTPEALSGVLLDEAFLDTLALLYNNPDQLRALLTLLSSDTAPRWMTVMRFYSECGDGSPAVYTCVDDLCRGYDLTRLSYGRSIFTEHVLGFELVPPSLFNVVVAIRNEATRTNRAVRLPVSTAAAPEGITLFYGLYNAVKEFCLRHQLDPPLLRHLDKYYAGLPPELKQTRVNLPAHSRYGPQAVDAR

SEQ ID NO: 46 - protein, 278 aa, Artificial Sequence
  gL G145L mutant
MCRRPDCGFSFSPGPVILLWCCLLLPIVSSAAVSVAPTAAEKVPAECPELTRRCLLGEVFEGDKYESWLRPLVNVTGRDGPLSQLIRYRPVTPEALSGVLLDEAFLDTLALLYNNPDQLRALLTLLSSDTAPRWMTVMRGYSECLDGSPAVYTCVDDLCRGYDLTRLSYGRSIFTEHVLGFELVPPSLFNVVVAIRNEATRTNRAVRLPVSTAAAPEGITLFYGLYNAVKEFCLRHQLDPPLLRHLDKYYAGLPPELKQTRVNLPAHSRYGPQAVDAR

SEQ ID NO: 47 - protein, 248 aa, Artificial Sequence
  mature gL G145L mutant
AAVSVAPTAAEKVPAECPELTRRCLLGEVFEGDKYESWLRPLVNVTGRDGPLSQLIRYRPVTPEALSGVLLDEAFLDTLALLYNNPDQLRALLTLLSSDTAPRWMTVMRGYSECLDGSPAVYTCVDDLCRGYDLTRLSYGRSIFTEHVLGFELVPPSLFNVVVAIRNEATRTNRAVRLPVSTAAAPEGITLFYGLYNAVKEFCLRHQLDPPLLRHLDKYYAGLPPELKQTRVNLPAHSRYGPQAVDAR

SEQ ID NO: 48 - protein, 278 aa, Artificial Sequence
  gL A150C mutant
MCRRPDCGFSFSPGPVILLWCCLLLPIVSSAAVSVAPTAAEKVPAECPELTRRCLLGEVFEGDKYESWLRPLVNVTGRDGPLSQLIRYRPVTPEALSGVLLDEAFLDTLALLYNNPDQLRALLTLLSSDTAPRWMTVMRGYSECGDGSPCVYTCVDDLCRGYDLTRLSYGRSIFTEHVLGFELVPPSLFNVVVAIRNEATRTNRAVRLPVSTAAAPEGITLFYGLYNAVKEFCLRHQLDPPLLRHLDKYYAGLPPELKQTRVNLPAHSRYGPQAVDAR

SEQ ID NO: 49 - protein, 248 aa, Artificial Sequence
  mature gL A150C mutant
AAVSVAPTAAEKVPAECPELTRRCLLGEVFEGDKYESWLRPLVNVTGRDGPLSQLIRYRPVTPEALSGVLLDEAFLDTLALLYNNPDQLRALLTLLSSDTAPRWMTVMRGYSECGDGSPCVYTCVDDLCRGYDLTRLSYGRSIFTEHVLGFELVPPSLFNVVVAIRNEATRTNRAVRLPVSTAAAPEGITLFYGLYNAVKEFCLRHQLDPPLLRHLDKYYAGLPPELKQTRVNLPAHSRYGPQAVDAR

SEQ ID NO: 50 - protein, 278 aa, Artificial Sequence
  gL R160C mutant
MCRRPDCGFSFSPGPVILLWCCLLLPIVSSAAVSVAPTAAEKVPAECPELTRRCLLGEVFEGDKYESWLRPLVNVTGRDGPLSQLIRYRPVTPEALSGVLLDEAFLDTLALLYNNPDQLRALLTLLSSDTAPRWMTVMRGYSECGDGSPAVYTCVDDLCCGYDLTRLSYGRSIFTEHVLGFELVPPSLFNVVVAIRNEATRTNRAVRLPVSTAAAPEGITLFYGLYNAVKEFCLRHQLDPPLLRHLDKYYAGLPPELKQTRVNLPAHSRYGPQAVDAR

SEQ ID NO: 51 - protein, 248 aa, Artificial Sequence
  mature gL R160C mutant
AAVSVAPTAAEKVPAECPELTRRCLLGEVFEGDKYESWLRPLVNVTGRDGPLSQLIRYRPVTPEALSGVLLDEAFLDTLALLYNNPDQLRALLTLLSSDTAPRWMTVMRGYSECGDGSPAVYTCVDDLCCGYDLTRLSYGRSIFTEHVLGFELVPPSLFNVVVAIRNEATRTNRAVRLPVSTAAAPEGITLFYGLYNAVKEFCLRHQLDPPLLRHLDKYYAGLPPELKQTRVNLPAHSRYGPQAVDAR

SEQ ID NO: 52 - protein, 278 aa, Artificial Sequence
  gL R166C mutant
MCRRPDCGFSFSPGPVILLWCCLLLPIVSSAAVSVAPTAAEKVPAECPELTRRCLLGEVFEGDKYESWLRPLVNVTGRDGPLSQLIRYRPVTPEALSGVLLDEAFLDTLALLYNNPDQLRALLTLLSSDTAPRWMTVMRGYSECGDGSPAVYTCVDDLCRGYDLTCLSYGRSIFTEHVLGFELVPPSLFNVVVAIRNEATRTNRAVRLPVSTAAAPEGITLFYGLYNAVKEFCLRHQLDPPLLRHLDKYYAGLPPELKQTRVNLPAHSRYGPQAVDAR

SEQ ID NO: 53 - protein, 248 aa, Artificial Sequence
  mature gL R166C mutant
AAVSVAPTAAEKVPAECPELTRRCLLGEVFEGDKYESWLRPLVNVTGRDGPLSQLIRYRPVTPEALSGVLLDEAFLDTLALLYNNPDQLRALLTLLSSDTAPRWMTVMRGYSECGDGSPAVYTCVDDLCRGYDLTCLSYGRSIFTEHVLGFELVPPSLFNVVVAIRNEATRTNRAVRLPVSTAAAPEGITLFYGLYNAVKEFCLRHQLDPPLLRHLDKYYAGLPPELKQTRVNLPAHSRYGPQAVDAR

SEQ ID NO: 54 - protein, 278 aa, Artificial Sequence
  gL C233V mutant
MCRRPDCGFSFSPGPVILLWCCLLLPIVSSAAVSVAPTAAEKVPAECPELTRRCLLGEVFEGDKYESWLRPLVNVTGRDGPLSQLIRYRPVTPEALSGVLLDEAFLDTLALLYNNPDQLRALLTLLSSDTAPRWMTVMRGYSECGDGSPAVYTCVDDLCRGYDLTRLSYGRSIFTEHVLGFELVPPSLFNVVVAIRNEATRTNRAVRLPVSTAAAPEGITLFYGLYNAVKEFVLRHQLDPPLLRHLDKYYAGLPPELKQTRVNLPAHSRYGPQAVDAR

SEQ ID NO: 55 - protein, 248 aa, Artificial Sequence
  mature gL C233V mutant
AAVSVAPTAAEKVPAECPELTRRCLLGEVFEGDKYESWLRPLVNVTGRDGPLSQLIRYRPVTPEALSGVLLDEAFLDTLALLYNNPDQLRALLTLLSSDTAPRWMTVMRGYSECGDGSPAVYTCVDDLCRGYDLTRLSYGRSIFTEHVLGFELVPPSLFNVVVAIRNEATRTNRAVRLPVSTAAAPEGITLFYGLYNAVKEFVLRHQLDPPLLRHLDKYYAGLPPELKQTRVNLPAHSRYGPQAVDAR

SEQ ID NO: 56 - protein, 171 aa, Artificial Sequence
  pUL128 M48C and G107C mutant
MSPKDLTPFLTTLWLLLGHSRVPRVRAEECCEFINVNHPPERCYDFKCCNRFTVALRCPDGEVCYSPEKTAEIRGIVTTMTHSLTRQVVHNKLTSCNYNPLYLEADCRIRCGKVNDKAQYLLGAAGSVPYRWINLEYDKITRIVGLDQYLESVKKHKRLDVCRAKMGYMLQ

SEQ ID NO: 57 - protein, 144 aa, Artificial Sequence
  mature pUL128 M48C and G107C mutant
EECCEFINVNHPPERCYDFKCCNRFTVALRCPDGEVCYSPEKTAEIRGIVTTMTHSLTRQVVHNKLTSCNYNPLYLEADCRIRCGKVNDKAQYLLGAAGSVPYRWINLEYDKITRIVGLDQYLESVKKHKRLDVCRAKMGYMLQ

SEQ ID NO: 58 - protein, 171 aa, Artificial Sequence
  pUL128 V77I mutant
MSPKDLTPFLTTLWLLLGHSRVPRVRAEECCEFINVNHPPERCYDFKMCNRFTVALRCPDGEVCYSPEKTAEIRGIITTMTHSLTRQVVHNKLTSCNYNPLYLEADGRIRCGKVNDKAQYLLGAAGSVPYRWINLEYDKITRIVGLDQYLESVKKHKRLDVCRAKMGYMLQ

SEQ ID NO: 59 - protein, 144 aa, Artificial Sequence
  mature pUL128 V77I mutant
EECCEFINVNHPPERCYDFKMCNRFTVALRCPDGEVCYSPEKTAEIRGIITTMTHSLTRQVVHNKLTSCNYNPLYLEADGRIRCGKVNDKAQYLLGAAGSVPYRWINLEYDKITRIVGLDQYLESVKKHKRLDVCRAKMGYMLQ

SEQ ID NO: 60 - protein, 171 aa, Artificial Sequence
  pUL128 S83C mutant
MSPKDLTPFLTTLWLLLGHSRVPRVRAEECCEFINVNHPPERCYDFKMCNRFTVALRCPDGEVCYSPEKTAEIRGIVTTMTHCLTRQVVHNKLTSCNYNPLYLEADGRIRCGKVNDKAQYLLGAAGSVPYRWINLEYDKITRIVGLDQYLESVKKHKRLDVCRAKMGYMLQ

SEQ ID NO: 61 - protein, 144 aa, Artificial Sequence
  mature pUL128 S83C mutant
EECCEFINVNHPPERCYDFKMCNRFTVALRCPDGEVCYSPEKTAEIRGIVTTMTHCLTRQVVHNKLTSCNYNPLYLEADGRIRCGKVNDKAQYLLGAAGSVPYRWINLEYDKITRIVGLDQYLESVKKHKRLDVCRAKMGYMLQ

SEQ ID NO: 62 - protein, 171 aa, Artificial Sequence
  pUL128 Y98C mutant
MSPKDLTPFLTTLWLLLGHSRVPRVRAEECCEFINVNHPPERCYDFKMCNRFTVALRCPDGEVCYSPEKTAEIRGIVTTMTHSLTRQVVHNKLTSCNCNPLYLEADGRIRCGKVNDKAQYLLGAAGSVPYRWINLEYDKITRIVGLDQYLESVKKHKRLDVCRAKMGYMLQ

SEQ ID NO: 63 - protein, 144 aa, Artificial Sequence
  mature pUL128 Y98C mutant
EECCEFINVNHPPERCYDFKMCNRFTVALRCPDGEVCYSPEKTAEIRGIVTTMTHSLTRQVVHNKLTSCNCNPLYLEADGRIRCGKVNDKAQYLLGAAGSVPYRWINLEYDKITRIVGLDQYLESVKKHKRLDVCRAKMGYMLQ

SEQ ID NO: 64 - protein, 171 aa, Artificial Sequence
  pUL128 L103I mutant
MSPKDLTPFLTTLWLLLGHSRVPRVRAEECCEFINVNHPPERCYDFKMCNRFTVALRCPDGEVCYSPEKTAEIRGIVTTMTHSLTRQVVHNKLTSCNYNPLYIEADGRIRCGKVNDKAQYLLGAAGSVPYRWINLEYDKITRIVGLDQYLESVKKHKRLDVCRAKMGYMLQ

SEQ ID NO: 65 - protein, 144 aa, Artificial Sequence
  mature pUL128 L103I mutant
EECCEFINVNHPPERCYDFKMCNRFTVALRCPDGEVCYSPEKTAEIRGIVTTMTHSLTRQVVHNKLTSCNYNPLYIEADGRIRCGKVNDKAQYLLGAAGSVPYRWINLEYDKITRIVGLDQYLESVKKHKRLDVCRAKMGYMLQ

SEQ ID NO: 66 - protein, 171 aa, Artificial Sequence
  pUL128 R142C mutant
MSPKDLTPFLTTLWLLLGHSRVPRVRAEECCEFINVNHPPERCYDFKMCNRFTVALRCPDGEVCYSPEKTAEIRGIVTTMTHSLTRQVVHNKLTSCNYNPLYLEADGRIRCGKVNDKAQYLLGAAGSVPYRWINLEYDKITCIVGLDQYLESVKKHKRLDVCRAKMGYMLQ

SEQ ID NO: 67 - protein, 144 aa, Artificial Sequence
  mature pUL128 R142C mutant
EECCEFINVNHPPERCYDFKMCNRFTVALRCPDGEVCYSPEKTAEIRGIVTTMTHSLTRQVVHNKLTSCNYNPLYLEADGRIRCGKVNDKAQYLLGAAGSVPYRWINLEYDKITCIVGLDQYLESVKKHKRLDVCRAKMGYMLQ

SEQ ID NO: 68 - protein, 214 aa, Artificial Sequence
  pUL130 Y56C mutant
MLRLLLRHHFHCLLLCAVWATPCLASPWSTLTANQNPSPPWSKLTYSKPHDAATFCCPFLYPSPPRSPLQFSGFQRVSTGPECRNETLYLLYNREGQTLVERSSTWVKKVIWYLSGRNQTILQRMPRTASKPSDGNVQISVEDAKIFGAHMVPKQTKLLRFVVNDGTRYQMCVMKLESWAHVFRDYSVSFQVRLTFTEANNQTYTFCTHPNLIV

SEQ ID NO: 69 - protein, 189 aa, Artificial Sequence
  mature pUL130 Y56C mutant
SPWSTLTANQNPSPPWSKLTYSKPHDAATFCCPFLYPSPPRSPLQFSGFQRVSTGPECRNETLYLLYNREGQTLVERSSTWVKKVIWYLSGRNQTILQRMPRTASKPSDGNVQISVEDAKIFGAHMVPKQTKLLRFVVNDGTRYQMCVMKLESWAHVFRDYSVSFQVRLTFTEANNQTYTFCTHPNLIV

SEQ ID NO: 70 - protein, 214 aa, Artificial Sequence
  pUL130 P62C mutant
MLRLLLRHHFHCLLLCAVWATPCLASPWSTLTANQNPSPPWSKLTYSKPHDAATFYCPFLYCSPPRSPLQFSGFQRVSTGPECRNETLYLLYNREGQTLVERSSTWVKKVIWYLSGRNQTILQRMPRTASKPSDGNVQISVEDAKIFGAHMVPKQTKLLRFVVNDGTRYQMCVMKLESWAHVFRDYSVSFQVRLTFTEANNQTYTFCTHPNLIV

SEQ ID NO: 71 - protein, 189 aa, Artificial Sequence
  mature pUL130 P62C mutant
SPWSTLTANQNPSPPWSKLTYSKPHDAATFYCPFLYCSPPRSPLQFSGFQRVSTGPECRNETLYLLYNREGQTLVERSSTWVKKVIWYLSGRNQTILQRMPRTASKPSDGNVQISVEDAKIFGAHMVPKQTKLLRFVVNDGTRYQMCVMKLESWAHVFRDYSVSFQVRLTFTEANNQTYTFCTHPNLIV

SEQ ID NO: 72 - protein, 214 aa, Artificial Sequence
  pUL130 P64C mutant
MLRLLLRHHFHCLLLCAVWATPCLASPWSTLTANQNPSPPWSKLTYSKPHDAATFYCPFLYPSCPRSPLQFSGFQRVSTGPECRNETLYLLYNREGQTLVERSSTWVKKVIWYLSGRNQTILQRMPRTASKPSDGNVQISVEDAKIFGAHMVPKQTKLLRFVVNDGTRYQMCVMKLESWAHVFRDYSVSFQVRLTFTEANNQTYTFCTHPNLIV

SEQ ID NO: 73 - protein, 189 aa, Artificial Sequence
  mature pUL130 P64C mutant
SPWSTLTANQNPSPPWSKLTYSKPHDAATFYCPFLYPSCPRSPLQFSGFQRVSTGPECRNETLYLLYNREGQTLVERSSTWVKKVIWYLSGRNQTILQRMPRTASKPSDGNVQISVEDAKIFGAHMVPKQTKLLRFVVNDGTRYQMCVMKLESWAHVFRDYSVSFQVRLTFTEANNQTYTFCTHPNLIV

SEQ ID NO: 74 - protein, 214 aa, Artificial Sequence
  pUL130 E95C mutant
MLRLLLRHHFHCLLLCAVWATPCLASPWSTLTANQNPSPPWSKLTYSKPHDAATFYCPFLYPSPPRSPLQFSGFQRVSTGPECRNETLYLLYNRCGQTLVERSSTWVKKVIWYLSGRNQTILQRMPRTASKPSDGNVQISVEDAKIFGAHMVPKQTKLLRFVVNDGTRYQMCVMKLESWAHVFRDYSVSFQVRLTFTEANNQTYTFCTHPNLIV

SEQ ID NO: 75 - protein, 189 aa, Artificial Sequence
  mature pUL130 E95C mutant
SPWSTLTANQNPSPPWSKLTYSKPHDAATFYCPFLYPSPPRSPLQFSGFQRVSTGPECRNETLYLLYNRCGQTLVERSSTWVKKVIWYLSGRNQTILQRMPRTASKPSDGNVQISVEDAKIFGAHMVPKQTKLLRFVVNDGTRYQMCVMKLESWAHVFRDYSVSFQVRLTFTEANNQTYTFCTHPNLIV

SEQ ID NO: 76 - protein, 214 aa, Artificial Sequence
  pUL130 T167C mutant
MLRLLLRHHFHCLLLCAVWATPCLASPWSTLTANQNPSPPWSKLTYSKPHDAATFYCPFLYPSPPRSPLQFSGFQRVSTGPECRNETLYLLYNREGQTLVERSSTWVKKVIWYLSGRNQTILQRMPRTASKPSDGNVQISVEDAKIFGAHMVPKQTKLLRFVVNDGCRYQMCVMKLESWAHVFRDYSVSFQVRLTFTEANNQTYTFCTHPNLIV

SEQ ID NO: 77 - protein, 189 aa, Artificial Sequence
  mature pUL130 T167C mutant
SPWSTLTANQNPSPPWSKLTYSKPHDAATFYCPFLYPSPPRSPLQFSGFQRVSTGPECRNETLYLLYNREGQTLVERSSTWVKKVIWYLSGRNQTILQRMPRTASKPSDGNVQISVEDAKIFGAHMVPKQTKLLRFVVNDGCRYQMCVMKLESWAHVFRDYSVSFQVRLTFTEANNQTYTFCTHPNLIV

SEQ ID NO: 78 - protein, 214 aa, Artificial Sequence
  pUL130 Y204C mutant
MLRLLLRHHFHCLLLCAVWATPCLASPWSTLTANQNPSPPWSKLTYSKPHDAATFYCPFLYPSPPRSPLQFSGFQRVSTGPECRNETLYLLYNREGQTLVERSSTWVKKVIWYLSGRNQTILQRMPRTASKPSDGNVQISVEDAKIFGAHMVPKQTKLLRFVVNDGTRYQMCVMKLESWAHVFRDYSVSFQVRLTFTEANNQTCTFCTHPNLIV

SEQ ID NO: 79 - protein, 189 aa, Artificial Sequence
  mature pUL130 Y204C mutant
SPWSTLTANQNPSPPWSKLTYSKPHDAATFYCPFLYPSPPRSPLQFSGFQRVSTGPECRNETLYLLYNREGQTLVERSSTWVKKVIWYLSGRNQTILQRMPRTASKPSDGNVQISVEDAKIFGAHMVPKQTKLLRFVVNDGTRYQMCVMKLESWAHVFRDYSVSFQVRLTFTEANNQTCTFCTHPNLIV

SEQ ID NO: 80 - protein, 129 aa, Artificial Sequence
  pUL131A Y52F and A67V mutant
MRLCRVWLSVCLCAVVLGQCQRETAEKNDYYRVPHYWDACSRALPDQTRYKFVEQLVDLTLNYHYDVSHGLDNFDVLKRINVTEVSLLISDFRRQNRRGGTNKRTTFNAAGSLAPHARSLEFSVRLFAN

SEQ ID NO: 81 - protein, 111 aa, Artificial Sequence
  mature pUL131A Y52F and A67V mutant
QCQRETAEKNDYYRVPHYWDACSRALPDQTRYKFVEQLVDLTLNYHYDVSHGLDNFDVLKRINVTEVSLLISDFRRQNRRGGTNKRTTFNAAGSLAPHARSLEFSVRLFAN

SEQ ID NO: 82 - protein, 129 aa, Artificial Sequence
  pUL131A S86F mutant
MRLCRVWLSVCLCAVVLGQCQRETAEKNDYYRVPHYWDACSRALPDQTRYKYVEQLVDLTLNYHYDASHGLDNFDVLKRINVTEVFLLISDFRRQNRRGGTNKRTTFNAAGSLAPHARSLEFSVRLFAN

SEQ ID NO: 83 - protein, 111 aa, Artificial Sequence
  mature pUL131A S86F mutant
QCQRETAEKNDYYRVPHYWDACSRALPDQTRYKYVEQLVDLTLNYHYDASHGLDNFDVLKRINVTEVFLLISDFRRQNRRGGTNKRTTFNAAGSLAPHARSLEFSVRLFAN